European Patent Application EP 4 417 190 A1, published August 21, 2024. Title: CYCLIC PEPTIDES WITH ANTIAGING EFFICACY. Applicant: LIPOTRUE, S.L. The sequence listing filed with the application follows.

SEQUENCE LISTING (2 sequences)

SEQ ID NO: 1 - protein, 6 aa, synthetic construct
  REGION 1..6: note = circular peptide; note (original language) = Peptido circular
WFRALH

SEQ ID NO: 2 - protein, 6 aa, synthetic construct
  REGION 1..6: note = Circular peptide; note (original language) = Peptido circular
FWHALR